European Patent Specification EP 3 864 156 B1, published August 16, 2023. Title: Plasmid containing a sequence encoding an mRNA with a segmented poly(A) tail. Applicant: ethris GmbH. The sequence listing filed with the application follows.

SEQUENCE LISTING (9 sequences)

SEQ ID NO: 1 - DNA, 34 bp, Artificial Sequence
  PCR primer forward / Oligo I
gtgactgctagctaatacgactcactatagggag

SEQ ID NO: 2 - DNA, 163 bp, Artificial Sequence
  PCR primer reverse / Oligo II
agtcacttcgaattttttttttttttttttttttttttttttttttttttttttttttttttttttttttttttttttttttttttttttttttttttttttttttttttttttttttttttttttttttttagatctttacacggcgatcttgccgcccttc

SEQ ID NO: 3 - DNA, 150 bp, Artificial Sequence
  PCR primer forward /Oligo I
gtgactagatctaaaaaaaaaaaaaaaaaaaaaaaaaaaaaaaaaaaaaaaaaaaaaaaaaaaaaaaaaaaaatgcataaaaaaaaaaaaaaaaaaaaaaaaaaaaaaaaaaaaaaaaaaaaaaaaaaaaaaaaaaaattcgaagtgact

SEQ ID NO: 4 - DNA, 150 bp, Artificial Sequence
  PCR primer reverse / Oligo II
agtcacttcgaattttttttttttttttttttttttttttttttttttttttttttttttttttttttttttatgcatttttttttttttttttttttttttttttttttttttttttttttttttttttttttttttagatctagtcac

SEQ ID NO: 5 - DNA, 156 bp, Artificial Sequence
  PCR primer forward / Oligo I
gtgactagatctaaaaaaaaaaaaaaaaaaaaaaaaaaaaaaaaaaaaaaaaatgcataaaaaaaaaaaaaaaaaaaaaaaaaaaaaaaaaaaaaaaagatatcaaaaaaaaaaaaaaaaaaaaaaaaaaaaaaaaaaaaaaaattcgaagtgact

SEQ ID NO: 6 - DNA, 156 bp, Artificial Sequence
  PCR primer reverse /Oligo II
agtcacttcgaattttttttttttttttttttttttttttttttttttttttgatatcttttttttttttttttttttttttttttttttttttttttatgcatttttttttttttttttttttttttttttttttttttttttagatctagtcac

SEQ ID NO: 7 - DNA, 164 bp, Artificial Sequence
  PCR primer reverse / Oligo II
agtcacttcgaattttttttttttttttttttttttttttttttttttttttttttttttttttttttttttgttttttttttttttttttttttttttttttttttttttttttttttttttttttttttttagatctttacacggcgatcttgccgcccttc

SEQ ID NO: 8 - DNA, 164 bp, Artificial Sequence
  PCR primer reverse / Oligo II
agtcacttcgaattttttttttttttttttttttttttttttttttttttttttttttttttttttttttttcttttttttttttttttttttttttttttttttttttttttttttttttttttttttttttagatctttacacggcgatcttgccgcccttc

SEQ ID NO: 9 - DNA, 164 bp, Artificial Sequence
  PCR primer reverse / Oligo II
agtcacttcgaattttttttttttttttttttttttttttttttttttttttttttttttttttttttttttattttttttttttttttttttttttttttttttttttttttttttttttttttttttttttagatctttacacggcgatcttgccgcccttc